European Patent Application EP 4 516 286 A1, published March 5, 2025. Title: TREHALOSE-BASED COMBINED THERAPY FOR LYSOSOMAL DAMAGE. Applicant: GENETHON. The sequence listing filed with the application follows.

SEQUENCE LISTING (4 sequences)

SEQ ID NO: 1 - DNA, 3594 bp, Homo sapiens
  source 1..3594: mol_type = genomic DNA
atgctttggtgggaagaagtagaggactgttatgaaagagaagatgttcaaaagaaaacattcacaaaatgggtaaatgcacaattttctaagtttgggaagcagcatattgagaacctcttcagtgacctacaggatgggaggcgcctcctagacctcctcgaaggcctgacagggcaaaaactgccaaaagaaaaaggatccacaagagttcatgccctgaacaatgtcaacaaggcactgcgggttttgcagaacaataatgttgatttagtgaatattggaagtactgacatcgtagatggaaatcataaactgactcttggtttgatttggaatataatcctccactggcaggtcaaaaatgtaatgaaaaatatcatggctggattgcaacaaaccaacagtgaaaagattctcctgagctgggtccgacaatcaactcgtaattatccacaggttaatgtaatcaacttcaccaccagctggtctgatggcctggctttgaatgctctcatccatagtcataggccagacctatttgactggaatagtgtggtttgccagcagtcagccacacaacgactggaacatgcattcaacatcgccagatatcaattaggcatagagaaactactcgatcctgaagatgttgataccacctatccagataagaagtccatcttaatgtacatcacatcactcttccaagttttgcctcaacaagtgagcattgaagccatccaggaagtggaaatgttgccaaggccacctaaagtgactaaagaagaacattttcagttacatcatcaaatgcactattctcaacagatcacggtcagtctagcacagggatatgagagaacttcttcccctaagcctcgattcaagagctatgcctacacacaggctgcttatgtcaccacctctgaccctacacggagcccatttccttcacagcatttggaagctcctgaagacaagtcatttggcagttcattgatggagagtgaagtaaacctggaccgttatcaaacagctttagaagaagtattatcgtggcttctttctgctgaggacacattgcaagcacaaggagagatttctaatgatgtggaagtggtgaaagaccagtttcatactcatgaggggtacatgatggatttgacagcccatcagggccgggttggtaatattctacaattgggaagtaagctgattggaacaggaaaattatcagaagatgaagaaactgaagtacaagagcagatgaatctcctaaattcaagatgggaatgcctcagggtagctagcatggaaaaacaaagcaatttacatagagttttaatggatctccagaatcagaaactgaaagagttgaatgactggctaacaaaaacagaagaaagaacaaggaaaatggaggaagagcctcttggacctgatcttgaagacctaaaacgccaagtacaacaacataaggtgcttcaagaagatctagaacaagaacaagtcagggtcaattctctcactcacatggtggtggtagttgatgaatctagtggagatcacgcaactgctgctttggaagaacaacttaaggtattgggagatcgatgggcaaacatctgtagatggacagaagaccgctgggttcttttacaagacatccttctcaaatggcaacgtcttactgaagaacagtgcctttttagtgcatggctttcagaaaaagaagatgcagtgaacaagattcacacaactggctttaaagatcaaaatgaaatgttatcaagtcttcaaaaactggccgttttaaaagcggatctagaaaagaaaaagcaatccatgggcaaactgtattcactcaaacaagatcttctttcaacactgaagaataagtcagtgacccagaagacggaagcatggctggataactttgcccggtgttgggataatttagtccaaaaacttgaaaagagtacagcacagatttcacaggctgtcaccaccactcagccatcactaacacagacaactgtaatggaaacagtaactacggtgaccacaagggaacagatcctggtaaagcatgctcaagaggaacttccaccaccacctccccaaaagaagaggcagattactgtggatacccttgaaagactccaggaacttcaagaggccacggatgagctggacctcaagctgcgccaagctgaggtgatcaagggatcctggcagcccgtgggcgatctcctcattgactctctccaagatcacctcgagaaagtcaaggcacttcgaggagaaattgcgcctctgaaagagaacgtgagccacgtcaatgaccttgctcgccagcttaccactttgggcattcagctctcaccgtataacctcagcactctggaagacctgaacaccagatggaagcttctgcaggtggccgtcgaggaccgagtcaggcagctgcatgaagcccacagggactttggtccagcatctcagcactttctttccacgtctgtccagggtccctgggagagagccatctcgccaaacaaagtgccctactatatcaaccacgagactcaaacaacttgctgggaccatcccaaaatgacagagctctaccagtctttagctgacctgaataatgtcagattctcagcttataggactgccatgaaactccgaagactgcagaaggccctttgcttggatctcttgagcctgtcagctgcatgtgatgccttggaccagcacaacctcaagcaaaatgaccagcccatggatatcctgcagattattaattgtttgaccactatttatgaccgcctggagcaagagcacaacaatttggtcaacgtccctctctgcgtggatatgtgtctgaactggctgctgaatgtttatgatacgggacgaacagggaggatccgtgtcctgtcttttaaaactggcatcatttccctgtgtaaagcacatttggaagacaagtacagataccttttcaagcaagtggcaagttcaacaggattttgtgaccagcgcaggctgggcctccttctgcatgattctatccaaattccaagacagttgggtgaagttgcatcctttgggggcagtaacattgagccaagtgtccggagctgcttccaatttgctaataataagccagagatcgaagcggccctcttcctagactggatgagactggaaccccagtccatggtgtggctgcccgtcctgcacagagtggctgctgcagaaactgccaagcatcaggccaaatgtaacatctgcaaagagtgtccaatcattggattcaggtacaggagtctaaagcactttaattatgacatctgccaaagctgctttttttctggtcgagttgcaaaaggccataaaatgcactatcccatggtggaatattgcactccgactacatcaggagaagatgttcgagactttgccaaggtactaaaaaacaaatttcgaaccaaaaggtattttgcgaagcatccccgaatgggctacctgccagtgcagactgtcttagagggggacaacatggaaactgacacaatgtga

SEQ ID NO: 2 - DNA, 1165 bp, Homo sapiens
  source 1..1165: mol_type = genomic DNA
catggctgagacactcttctggactcctctcctcgtggttctcctggcagggctgggggacaccgaggcccagcagaccacgctacacccacttgtgggccgtgtctttgtgcacaccttggaccatgagacgtttctgagccttcctgagcatgtcgctgtcccacccgctgtccacatcacctaccacgcccacctccagggacacccagacctgccccggtggctccgctacacccagcgcagcccccaccaccctggcttcctctacggctctgccaccccagaagatcgtgggctccaggtcattgaggtcacagcctacaatcgggacagctttgataccactcggcagaggctggtgctggagattggggacccagaaggccccctgctgccataccaagccgagttcctggtgcgcagccacgatgcggaggaggtgctgccctcaacacctgccagccgcttcctctcagccttggggggactctgggagcccggagagcttcagctgctcaacgtcacctctgccttggaccgtgggggccgtgtcccccttcccattgagggccgaaaagaaggggtatacattaaggtgggttctgcctcacctttttctacttgcctgaagatggtggcatcccccgatagccacgcccgctgtgcccagggccagcctccacttctgtcttgctacgacaccttggcaccccacttccgcgttgactggtgcaatgtgaccctggtggataagtcagtgccggagcctgcagatgaggtgcccaccccaggtgatgggatcctggagcatgacccgttcttctgcccacccactgaggccccagaccgtgacttcttggtggatgctctggtcaccctcctggtgcccctgctggtggccctgcttctcaccttgctgctggcctatgtcatgtgctgccggcgggagggaaggctgaagagagacctggctacctccgacatccagatggtccaccactgcaccatccacgggaacacagaggagctgcggcagatggcggccagccgcgaggtgccccggccactctccaccctgcccatgttcaatgtgcacacaggtgagcggctgcctccccgcgtggacagcgcccaggtgcccctcattctggaccagcactga

SEQ ID NO: 3 - DNA, 1164 bp, Homo sapiens
  source 1..1164: mol_type = genomic DNA
tcagtgctggtccaggatcaggggcacctgggcagagtccaccctggggggcagcctctcccctgtgtgcacattgaacatgggcagggtgctcaggggcctgggcacctccctgctggcagccatctgcctcagctcctctgtgttgccatggatggtgcagtggtgcaccatctggatgtcagaggtggccaggtccctcttcagcctgccctccctcctgcagcacatcacataggccagcagcagggtcagcagcagggccaccagcaggggcaccagcagggtgaccagggcatccaccaggaagtccctgtcaggggcctctgtgggggggcagaagaaggggtcatgctccaggatgccatccccaggggtgggcacctcatcagcaggctcaggcacagacttgtccaccagggtcacattgcaccagtccaccctgaagtggggggccagggtgtcatagcagctcagcagggggggctggccctgggcacacctggcatggctgtcagggctggccaccatcttcaggcaggtgctgaaggggctggcagagcccaccttgatgtacaccccctccttcctgccctcaatgggcaggggcaccctgccccccctgtccagggcagaggtcacattcagcagctgcagctccccaggctcccacaggccccccagggcagacaggaacctgctggcaggggtgctgggcagcacctcctcagcatcatggctcctgaccaggaactcagcctggtagggcagcagggggccctcagggtccccaatctccagcaccagcctctgcctggtggtgtcaaagctgtccctgttgtaggctgtcacctcaatcacttgcaggcccctgtcctcaggggtggcagagccatacaggaagccagggtggtgggggctcctctgggtgtacctcagccacctgggcaggtcagggtggccctgcaggtgggcatggtaggtgatgtgcacagcagggggcacagccacatgctcaggcaggctcaggaaggtctcatggtccagggtgtgcacaaacaccctgcccaccagggggtgcagggtggtctgctgggcctctgtgtcccccaggccagccagcagcaccaccagcaggggggtccagaacagggtctcagccat

SEQ ID NO: 4 - DNA, 1488 bp, Homo sapiens
  source 1..1488: mol_type = genomic DNA
atgagactgaccaggtgccaggctgccctggctgctgccatcaccctgaacctgctggtgctgttctatgtgagctggctgcagcaccagcccaggaacagcagggccaggggccccaggagggcctctgctgctggccccagggtgacagtgctggtgagggagtttgaggcctttgacaatgctgtgcctgagctggtggacagcttcctgcagcaggaccctgcccagcctgtggtggtggctgctgataccctgccctacccccccctggccctgcccaggatccccaatgtgaggctggccctgctgcagcctgccctggacaggcctgctgctgccagcaggcctgagacctatgtggccacagagtttgtggccctggtgcctgatggggccagggctgaggcccctggcctgctggagaggatggtggaggccctgagggctggctctgccaggctggtggctgcccctgtggccacagccaaccctgccaggtgcctggccctgaatgtgagcctgagagagtggacagccaggtatggggctgcccctgctgcccccaggtgtgatgccctggatggagatgctgtggtgctgctgagggccagggacctgttcaacctgtctgcccccctggccaggcctgtggggaccagcctgtttctgcagacagccctgaggggctgggctgtgcagctgctggacctgacctttgctgctgccaggcagccccccctggctacagcccacgccaggtggaaggctgagagggagggcagggccaggagggctgccctgctgagggccctggggatcaggctggtgagctgggaggggggcaggctggagtggtttggctgcaacaaggagacaaccaggtgctttgggacagtggtgggggatacccctgcctacctgtatgaggagaggtggacccccccctgctgcctgagggccctgagggagacagccaggtatgtggtgggggtgctggaggctgctggggtgaggtactggctggaggggggcagcctgctgggggctgccaggcacggggacattatcccctgggactatgatgtggacctgggcatctacctggaggatgtgggcaactgtgagcagctgaggggggctgaggctggctctgtggtggatgagaggggctttgtgtgggagaaggctgtggagggggactttttcagggtgcagtactctgagagcaaccacctgcacgtggacctgtggcccttctaccccaggaatggggtgatgaccaaggacacctggctggaccacaggcaggatgtggagttccctgagcacttcctgcagcccctggtgcccctgccctttgctggctttgtggcccaggcccccaacaactacaggaggttcctggagctgaagtttggccctggggtgattgagaacccccagtaccccaaccctgccctgctgagcctgacaggctctggctga